European Patent Specification EP 3 721 916 B1, published September 27, 2023. Title: Pretreatment composition for dental therapy and Kit for dental tissue generation. Applicant: National Center for Geriatrics and Gerontology. The sequence listing filed with the application follows.

SEQUENCE LISTING (40 sequences)

SEQ ID NO: 1 - DNA, 20 bp, Artificial Sequence
  primer
ggacttcgagcaagagatgg

SEQ ID NO: 2 - DNA, 20 bp, Artificial Sequence
  primer
agcactgtgttggcgtacag

SEQ ID NO: 3 - DNA, 21 bp, Artificial Sequence
  primer
gaaggtccctcagacatcccc

SEQ ID NO: 4 - DNA, 21 bp, Artificial Sequence
  primer
ccctgtaggaccttcggtgac

SEQ ID NO: 5 - DNA, 21 bp, Artificial Sequence
  primer
ttctgtggctgctgctcatag

SEQ ID NO: 6 - DNA, 20 bp, Artificial Sequence
  primer
gctctctagtcgctgaaggg

SEQ ID NO: 7 - DNA, 22 bp, Artificial Sequence
  primer
ctgtactccctggtgttcactg

SEQ ID NO: 8 - DNA, 21 bp, Artificial Sequence
  primer
ggttgagcaggtagatgttgg

SEQ ID NO: 9 - DNA, 20 bp, Artificial Sequence
  primer
caagtcgcagatcttgagca

SEQ ID NO: 10 - DNA, 20 bp, Artificial Sequence
  primer
cacttgcttgaagtcgatgc

SEQ ID NO: 11 - DNA, 21 bp, Artificial Sequence
  primer
ttctgtggctgctgctcatag

SEQ ID NO: 12 - DNA, 20 bp, Artificial Sequence
  primer
gctctctagtcgctgaaggg

SEQ ID NO: 13 - DNA, 22 bp, Artificial Sequence
  primer
ctgtactccctggtgttcactg

SEQ ID NO: 14 - DNA, 21 bp, Artificial Sequence
  primer
ggttgagcaggtagatgttgg

SEQ ID NO: 15 - DNA, 21 bp, Artificial Sequence
  primer
gaaggtccctcagacatcccc

SEQ ID NO: 16 - DNA, 21 bp, Artificial Sequence
  primer
ccctgtaggaccttcggtgac

SEQ ID NO: 17 - DNA, 20 bp, Artificial Sequence
  primer
aggccttggaactcaaggat

SEQ ID NO: 18 - DNA, 20 bp, Artificial Sequence
  primer
ccctttttggacttcaggtg

SEQ ID NO: 19 - DNA, 20 bp, Artificial Sequence
  primer
ccaggagcccagctatgaac

SEQ ID NO: 20 - DNA, 19 bp, Artificial Sequence
  primer
cccagggagaaggcaactg

SEQ ID NO: 21 - DNA, 22 bp, Artificial Sequence
  primer
ggccctaaacagatgaagtgct

SEQ ID NO: 22 - DNA, 16 bp, Artificial Sequence
  primer
tgccgccatccagagg

SEQ ID NO: 23 - DNA, 20 bp, Artificial Sequence
  primer
ttggcagccttcctgatttc

SEQ ID NO: 24 - DNA, 16 bp, Artificial Sequence
  primer
tgccgccatccagagg

SEQ ID NO: 25 - DNA, 20 bp, Artificial Sequence
  primer
accaggccgtgatctctatg

SEQ ID NO: 26 - DNA, 19 bp, Artificial Sequence
  primer
tccctttgtccctggtctc

SEQ ID NO: 27 - DNA, 21 bp, Artificial Sequence
  primer
gaaggtccctcagacatcccc

SEQ ID NO: 28 - DNA, 21 bp, Artificial Sequence
  primer
ccctgtaggaccttcggtgac

SEQ ID NO: 29 - DNA, 20 bp, Artificial Sequence
  primer
aaacatccgaggacaaggtg

SEQ ID NO: 30 - DNA, 20 bp, Artificial Sequence
  primer
cgtgtacaagtctgcgtcct

SEQ ID NO: 31 - DNA, 20 bp, Artificial Sequence
  primer
atacaggcggaaccacactc

SEQ ID NO: 32 - DNA, 19 bp, Artificial Sequence
  primer
gcctggggtccacagtaat

SEQ ID NO: 33 - DNA, 20 bp, Artificial Sequence
  primer
gccccagtcacctgctgtta

SEQ ID NO: 34 - DNA, 20 bp, Artificial Sequence
  primer
tccaggtggtccatggaatc

SEQ ID NO: 35 - DNA, 20 bp, Artificial Sequence
  primer
tggtggtgatgggcgtatct

SEQ ID NO: 36 - DNA, 20 bp, Artificial Sequence
  primer
ctggccatcactgctcaaag

SEQ ID NO: 37 - DNA, 20 bp, Artificial Sequence
  primer
cctcaggaagcttgaacctg

SEQ ID NO: 38 - DNA, 20 bp, Artificial Sequence
  primer
gggaaacctagggtgtggat

SEQ ID NO: 39 - DNA, 19 bp, Artificial Sequence
  primer
gacggaaagatgtggtgtg

SEQ ID NO: 40 - DNA, 23 bp, Artificial Sequence
  primer
aagacggaagttcttggtgtagg